European Patent Application EP 4 122 957 A1, published January 25, 2023. Title: ANGIOPOIETIN-LIKE 4 ANTIBODIES AND METHODS OF USE. Applicant: NOVARTIS AG. Application PCT/IB2015/055986. The sequence listing filed with the application follows.

SEQUENCE LISTING (233 sequences)

SEQ ID NO: 1 - protein, 406 aa, Homo sapiens
MSGAPTAGAALMLCAATAVLLSAQGGPVQSKSPRFASWDEMNVLAHGLLQLGQGLREHAERTRSQLSALERRLSACGSACQGTEGSTDLPLAPESRVDPEVLHSLQTQLKAQNSRIQQLFHKVAQQQRHLEKQHLRIQHLQSQFGLLDHKHLDHEVAKPARRKRLPEMAQPVDPAHNVSRLHRLPRDCQELFQVGERQSGLFEIQPQGSPPFLVNCKMTSDGGWTVIQRRHDGSVDFNRPWEAYKAGFGDPHGEFWLGLEKVHSITGDRNSRLAVQLRDWDGNAELLQFSVHLGGEDTAYSLQLTAPVAGQLGATTVPPSGLSVPFSTWDQDHDLRRDKNCAKSLSGGWWFGTCSHSNLNGQYFRSIPQQRQKLKKGIFWKTWRGRYYPLQATTMLIQPMAAEAAS

SEQ ID NO: 2 - DNA, 1225 bp, Homo sapiens
atgagcggtgctccgacggccggggcagccctgatgctctgcgccgccaccgccgtgctactgagcgctcagggcggacccgtgcagtccaagtcgccgcgctttgcgtcctgggacgagatgaatgtcctggcgcacggactcctgcagctcggccaggggctgcgcgaacacgcggagcgcacccgcagtcagctgagcgcgctggagcggcgcctgagcgcgtgcgggtccgcctgtcagggaaccgaggggtccaccgacctcccgttagcccctgagagccgggtggaccctgaggtccttcacagcctgcagacacaactcaaggctcagaacagcaggatccagcaactcttccacaaggtggcccagcagcagcggcacctggagaagcagcacctgcgaattcagcatctgcaaagccagtttggcctcctggaccacaagcacctagaccatgaggtggccaagcctgcccgaagaaagaggctgcccgagatggcccagccagttgacccggctcacaatgtcagccgcctgcaccggctgcccagggattgccaggagctgttccaggttggggagaggcagagtggactatttgaaatccagcctcaggggtctccgccatttttggtgaactgcaagatgacctcagatggaggctggacagtaattcagaggcgccacgatggctcagtggacttcaaccggccctgggaagcctacaaggcggggtttggggatccccacggcgagttctggctgggtctggagaaggtgcatagcatcacgggggaccgcaacagccgcctggccgtgcagctgcgggactgggatggcaacgccgagttgctgcagttctccgtgcacctgggtggcgaggacacggcctatagcctgcagctcactgcacccgtggccggccagctgggcgccaccaccgtcccacccagcggcctctccgtacccttctccacttgggaccaggatcacgacctccgcagggacaagaactgcgccaagagcctctctggaggctggtggtttggcacctgcagccattccaacctcaacggccagtacttccgctccatcccacagcagcggcagaagcttaagaagggaatcttctggaagacctggcggggccgctactacccgctgcaggccaccaccatgttgatccagcccatggcagcagaggcagcctcctagcgtc

SEQ ID NO: 3 - protein, 406 aa, Macaca fascicularis
MRGAPTAGAALMLCVATAVLLRAQGGPVQSKSPRFASWDEMNVLAHGLLQLGQGLREHAERTRSQLNALERRLSACGSACQGTEGSTALPLAPESRVDPEVLHSLQTQLKAQNSRIQQLFHKVAQQQRHLEKQHLRIQRLQSQVGLLDPKHLDHEVAKPARRKRRPEMAQPVDSAHNASRLHRLPRDCQELFEDGERQSGLFEIQPQGSPPFLVNCKMTSDGGWTVIQRRHDGSVDFNRPWEAYKAGFGDPQGEFWLGLEKVHSITGDRNSRLAVQLQDWDGNAESLQFSVHLGGEDTAYSLQLTEPVASQLGATTVPPSGLSVPFSTWDQDHDLRRDKNCAKSLSGGWWFGTCSHSNLNGQYFRSIPQQRQELKKGIFWKTWRGRYYPLQATTMLIQPTAAEAAS

SEQ ID NO: 4 - DNA, 1221 bp, Macaca fascicularis
atgcgcggtgctccgacggccggagcagccctgatgctctgcgtcgccacggccgtgctgctgagagctcagggcggcccggtgcagtccaagtctccgcgctttgcgtcctgggacgagatgaatgtcctggcgcacggactcctgcagctaggccaggggctgcgcgaacacgcggagcgcacccgcagtcagctgaacgcgctggagcggcgcctcagcgcttgcgggtctgcctgccagggaaccgaggggtccaccgccctcccgttagcccctgagagccgggtggaccctgaggtccttcacagcctgcagacacaactcaaggctcagaacagcaggatccagcaactcttccacaaggtggcccagcagcagcggcacctggagaagcagcacctgcgaattcagcgtctgcaaagccaggttggcctcctggaccccaagcacctagaccatgaggtggccaagcctgcccgaagaaagaggcggcccgagatggcccagccagttgactcggctcacaatgccagccgcctgcaccggctgcccagggattgccaggagctgtttgaagatggggagaggcagagtggactatttgagatccagcctcaggggtctccgccatttttggtgaactgcaagatgacctcagatggaggctggacagtaattcagaggcgccacgatggctctgtggacttcaaccggccctgggaagcctacaaggcggggtttggggatccccaaggcgagttctggctgggcctggagaaggtgcatagcatcacaggggaccgcaacagccgcctggccgtgcagctgcaggactgggatggcaacgccgagtcgctgcagttctctgtgcacctgggtggcgaggacacggcttacagcctgcagctcaccgagcccgtggccagccagttgggtgccaccaccgtcccgcctagcggcctctccgtacccttctccacttgggaccaggatcacgacctccgcagggacaagaactgcgccaagagcctctctggaggctggtggtttggcacctgcagccattccaacctcaatggccagtacttccgctccatcccacagcagcggcaggagcttaagaaaggaatcttctggaagacctggcggggccgctactacccgctgcaggccaccaccatgttgatccagcccacggcggcagaggcagcctcctag

SEQ ID NO: 5 - protein, 460 aa, Homo sapiens
MFTIKLLLFIVPLVISSRIDQDNSSFDSLSPEPKSRFAMLDDVKILANGLLQLGHGLKDFVHKTKGQINDIFQKLNIFDQSFYDLSLQTSEIKEEEKELRRTTYKLQVKNEEVKNMSLELNSKLESLLEEKILLQQKVKYLEEQLTNLIQNQPETPEHPEVTSLKTFVEKQDNSIKDLLQTVEDQYKQLNQQHSQIKEIENQLRRTSIQEPTEISLSSKPRAPRTTPFLQLNEIRNVKHDGIPAECTTIYNRGEHTSGMYAIRPSNSQVFHVYCDVISGSPWTLIQHRIDGSQNFNETWENYKYGFGRLDGEFWLGLEKIYSIVKQSNYVLRIELEDWKDNKHYIEYSFYLGNHETNYTLHLVAITGNVPNAIPENKDLVFSTWDHKAKGHFNCPEGYSGGWWWHDECGENNLNGKYNKPRAKSKPERRRGLSWKSQNGRLYSIKSTKMLIHPTDSESFE

SEQ ID NO: 6 - DNA, 1380 bp, Homo sapiens
atgttcacaattaagctccttctttttattgttcctctagttatttcctccagaattgatcaagacaattcatcatttgattctctatctccagagccaaaatcaagatttgctatgttagacgatgtaaaaattttagccaatggcctccttcagttgggacatggtcttaaagactttgtccataagacgaagggccaaattaatgacatatttcaaaaactcaacatatttgatcagtctttttatgatctatcgctgcaaaccagtgaaatcaaagaagaagaaaaggaactgagaagaactacatataaactacaagtcaaaaatgaagaggtaaagaatatgtcacttgaactcaactcaaaacttgaaagcctcctagaagaaaaaattctacttcaacaaaaagtgaaatatttagaagagcaactaactaacttaattcaaaatcaacctgaaactccagaacacccagaagtaacttcacttaaaacttttgtagaaaaacaagataatagcatcaaagaccttctccagaccgtggaagaccaatataaacaattaaaccaacagcatagtcaaataaaagaaatagaaaatcagctcagaaggactagtattcaagaacccacagaaatttctctatcttccaagccaagagcaccaagaactactccctttcttcagttgaatgaaataagaaatgtaaaacatgatggcattcctgctgaatgtaccaccatttataacagaggtgaacatacaagtggcatgtatgccatcagacccagcaactctcaagtttttcatgtctactgtgatgttatatcaggtagtccatggacattaattcaacatcgaatagatggatcacaaaacttcaatgaaacgtgggagaactacaaatatggttttgggaggcttgatggagaattttggttgggcctagagaagatatactccatagtgaagcaatctaattatgttttacgaattgagttggaagactggaaagacaacaaacattatattgaatattctttttacttgggaaatcacgaaaccaactatacgctacatctagttgcgattactggcaatgtccccaatgcaatcccggaaaacaaagatttggtgttttctacttgggatcacaaagcaaaaggacacttcaactgtccagagggttattcaggaggctggtggtggcatgatgagtgtggagaaaacaacctaaatggtaaatataacaaaccaagagcaaaatctaagccagagaggagaagaggattatcttggaagtctcaaaatggaaggttatactctataaaatcaaccaaaatgttgatccatccaacagattcagaaagctttgaa

SEQ ID NO: 7 - protein, 5 aa, Artificial Sequence
  source: /note="Description of Artificial Sequence: Synthetic peptide"
SSWMQ

SEQ ID NO: 8 - protein, 17 aa, Artificial Sequence
  source: /note="Description of Artificial Sequence: Synthetic peptide"
EIDPSDNYANYNQKFQG

SEQ ID NO: 9 - protein, 10 aa, Artificial Sequence
  source: /note="Description of Artificial Sequence: Synthetic peptide"
GSYFSNFFDY

SEQ ID NO: 10 - protein, 7 aa, Artificial Sequence
  source: /note="Description of Artificial Sequence: Synthetic peptide"
AYTFTSS

SEQ ID NO: 11 - protein, 6 aa, Artificial Sequence
  source: /note="Description of Artificial Sequence: Synthetic peptide"
DPSDNY

SEQ ID NO: 12 - protein, 10 aa, Artificial Sequence
  source: /note="Description of Artificial Sequence: Synthetic peptide"
GSYFSNFFDY

SEQ ID NO: 13 - protein, 119 aa, Artificial Sequence
  source: /note="Description of Artificial Sequence: Synthetic polypeptide"
QVQLVQSGAEVKKPGASVKVSCKASAYTFTSSWMQWVRQAPGQGLEWMGEIDPSDNYANYNQKFQGRVTLTVDTSTSTAYMELSSLRSEDTAVYYCASGSYFSNFFDYWGQGTLVTVSS

SEQ ID NO: 14 - DNA, 357 bp, Artificial Sequence
  source: /note="Description of Artificial Sequence: Synthetic polynucleotide"
caggtgcagctggtgcagtctggcgccgaagtgaagaaaccaggcgccagcgtgaaggtgtcctgcaaggccagcgcctacacctttaccagcagctggatgcagtgggtgcgccaggctcctggacagggcctggaatggatgggcgagatcgaccccagcgacaactacgccaactacaaccagaaattccagggcagagtgaccctgaccgtggacaccagcacctccaccgcctacatggaactgagcagcctgcggagcgaggacaccgccgtgtactattgtgccagcggcagctacttcagcaacttcttcgactactggggccagggcaccctcgtgaccgtgtcatct

SEQ ID NO: 15 - protein, 449 aa, Artificial Sequence
  source: /note="Description of Artificial Sequence: Synthetic polypeptide"
QVQLVQSGAEVKKPGASVKVSCKASAYTFTSSWMQWVRQAPGQGLEWMGEIDPSDNYANYNQKFQGRVTLTVDTSTSTAYMELSSLRSEDTAVYYCASGSYFSNFFDYWGQGTLVTVSSASTKGPSVFPLAPSSKSTSGGTAALGCLVKDYFPEPVTVSWNSGALTSGVHTFPAVLQSSGLYSLSSVVTVPSSSLGTQTYICNVNHKPSNTKVDKRVEPKSCDKTHTCPPCPAPELLGGPSVFLFPPKPKDTLMISRTPEVTCVVVDVSHEDPEVKFNWYVDGVEVHNAKTKPREEQYNSTYRVVSVLTVLHQDWLNGKEYKCKVSNKALPAPIEKTISKAKGQPREPQVYTLPPSREEMTKNQVSLTCLVKGFYPSDIAVEWESNGQPENNYKTTPPVLDSDGSFFLYSKLTVDKSRWQQGNVFSCSVMHEALHNHYTQKSLSLSPGK

SEQ ID NO: 16 - DNA, 1347 bp, Artificial Sequence
  source: /note="Description of Artificial Sequence: Synthetic polynucleotide"
caggtgcagctggtgcagtctggcgccgaagtgaagaaaccaggcgccagcgtgaaggtgtcctgcaaggccagcgcctacacctttaccagcagctggatgcagtgggtgcgccaggctcctggacagggcctggaatggatgggcgagatcgaccccagcgacaactacgccaactacaaccagaaattccagggcagagtgaccctgaccgtggacaccagcacctccaccgcctacatggaactgagcagcctgcggagcgaggacaccgccgtgtactattgtgccagcggcagctacttcagcaacttcttcgactactggggccagggcaccctcgtgaccgtgtcatctgctagcaccaagggccccagcgtgttccccctggcccccagcagcaagagcaccagcggcggcacagccgccctgggctgcctggtgaaggactacttccccgagcccgtgaccgtgtcctggaacagcggagccctgacctccggcgtgcacaccttccccgccgtgctgcagagcagcggcctgtacagcctgtccagcgtggtgacagtgcccagcagcagcctgggcacccagacctacatctgcaacgtgaaccacaagcccagcaacaccaaggtggacaagagagtggagcccaagagctgcgacaagacccacacctgccccccctgcccagccccagagctgctgggcggaccctccgtgttcctgttcccccccaagcccaaggacaccctgatgatcagcaggacccccgaggtgacctgcgtggtggtggacgtgagccacgaggacccagaggtgaagttcaactggtacgtggacggcgtggaggtgcacaacgccaagaccaagcccagagaggagcagtacaacagcacctacagggtggtgtccgtgctgaccgtgctgcaccaggactggctgaacggcaaggaatacaagtgcaaggtctccaacaaggccctgccagcccccatcgaaaagaccatcagcaaggccaagggccagccacgggagccccaggtgtacaccctgcccccctcccgggaggagatgaccaagaaccaggtgtccctgacctgtctggtgaagggcttctaccccagcgacatcgccgtggagtgggagagcaacggccagcccgagaacaactacaagaccacccccccagtgctggacagcgacggcagcttcttcctgtacagcaagctgaccgtggacaagtccaggtggcagcagggcaacgtgttcagctgcagcgtgatgcacgaggccctgcacaaccactacacccagaagagcctgagcctgtcccccggcaag

SEQ ID NO: 17 - protein, 11 aa, Artificial Sequence
  source: /note="Description of Artificial Sequence: Synthetic peptide"
KASQDIGSNLN

SEQ ID NO: 18 - protein, 7 aa, Artificial Sequence
  source: /note="Description of Artificial Sequence: Synthetic peptide"
AVSNRGP

SEQ ID NO: 19 - protein, 9 aa, Artificial Sequence
  source: /note="Description of Artificial Sequence: Synthetic peptide"
LQYASSPWT

SEQ ID NO: 20 - protein, 7 aa, Artificial Sequence
  source: /note="Description of Artificial Sequence: Synthetic peptide"
SQDIGSN

SEQ ID NO: 21 - protein, 3 aa, Artificial Sequence
  source: /note="Description of Artificial Sequence: Synthetic peptide"
AVS

SEQ ID NO: 22 - protein, 6 aa, Artificial Sequence
  source: /note="Description of Artificial Sequence: Synthetic peptide"
YASSPW

SEQ ID NO: 23 - protein, 107 aa, Artificial Sequence
  source: /note="Description of Artificial Sequence: Synthetic polypeptide"
EIVMTQSPATLSVSPGERATLSCKASQDIGSNLNWLQQKPGQAPRRLIYAVSNRGPGIPARFSGSRSGSEYTLTISSLQSEDFAVYYCLQYASSPWTFGQGTKVEIK

SEQ ID NO: 24 - DNA, 321 bp, Artificial Sequence
  source: /note="Description of Artificial Sequence: Synthetic polynucleotide"
gagatcgtgatgacacagagccccgccaccctgtccgtgtctccaggcgaaagagccaccctgagctgcaaagccagccaggacatcggcagcaacctgaactggctgcagcagaaaccaggccaggcccccagaaggctgatctacgctgtttccaaccgtggtcctggcatccccgccagattttccggcagcagatccggcagcgagtacaccctgaccatcagcagcctgcagagcgaggacttcgccgtgtactactgcctgcagtacgccagcagcccctggacatttggccagggcaccaaggtggaaatcaag

SEQ ID NO: 25 - protein, 214 aa, Artificial Sequence
  source: /note="Description of Artificial Sequence: Synthetic polypeptide"
EIVMTQSPATLSVSPGERATLSCKASQDIGSNLNWLQQKPGQAPRRLIYAVSNRGPGIPARFSGSRSGSEYTLTISSLQSEDFAVYYCLQYASSPWTFGQGTKVEIKRTVAAPSVFIFPPSDEQLKSGTASVVCLLNNFYPREAKVQWKVDNALQSGNSQESVTEQDSKDSTYSLSSTLTLSKADYEKHKVYACEVTHQGLSSPVTKSFNRGEC

SEQ ID NO: 26 - DNA, 642 bp, Artificial Sequence
  source: /note="Description of Artificial Sequence: Synthetic polynucleotide"
gagatcgtgatgacacagagccccgccaccctgtccgtgtctccaggcgaaagagccaccctgagctgcaaagccagccaggacatcggcagcaacctgaactggctgcagcagaaaccaggccaggcccccagaaggctgatctacgctgtttccaaccgtggtcctggcatccccgccagattttccggcagcagatccggcagcgagtacaccctgaccatcagcagcctgcagagcgaggacttcgccgtgtactactgcctgcagtacgccagcagcccctggacatttggccagggcaccaaggtggaaatcaagcgtacggtggccgctcccagcgtgttcatcttcccccccagcgacgagcagctgaagagcggcaccgccagcgtggtgtgcctgctgaacaacttctacccccgggaggccaaggtgcagtggaaggtggacaacgccctgcagagcggcaacagccaggagagcgtcaccgagcaggacagcaaggactccacctacagcctgagcagcaccctgaccctgagcaaggccgactacgagaagcataaggtgtacgcctgcgaggtgacccaccagggcctgtccagccccgtgaccaagagcttcaacaggggcgagtgc

SEQ ID NO: 27 - DNA, 357 bp, Artificial Sequence
  source: /note="Description of Artificial Sequence: Synthetic polynucleotide"
caggtgcagctggtgcagtcaggcgccgaagtgaagaaacccggcgctagtgtgaaagtcagctgtaaagctagtgcctacaccttcacctctagctggatgcagtgggtcagacaggccccaggtcagggcctggagtggatgggcgagatcgaccctagcgataactacgctaactataatcagaagtttcagggtagagtcaccctgaccgtggacactagcactagcaccgcctatatggaactgtctagcctgagatcagaggacaccgccgtctactactgcgctagtggtagctacttctctaacttcttcgactactggggtcagggcaccctggtcaccgtgtctagc

SEQ ID NO: 28 - protein, 449 aa, Artificial Sequence
  source: /note="Description of Artificial Sequence: Synthetic polypeptide"
QVQLVQSGAEVKKPGASVKVSCKASAYTFTSSWMQWVRQAPGQGLEWMGEIDPSDNYANYNQKFQGRVTLTVDTSTSTAYMELSSLRSEDTAVYYCASGSYFSNFFDYWGQGTLVTVSSASTKGPSVFPLAPSSKSTSGGTAALGCLVKDYFPEPVTVSWNSGALTSGVHTFPAVLQSSGLYSLSSVVTVPSSSLGTQTYICNVNHKPSNTKVDKRVEPKSCDKTHTCPPCPAPEAAGGPSVFLFPPKPKDTLMISRTPEVTCVVVDVSHEDPEVKFNWYVDGVEVHNAKTKPREEQYNSTYRVVSVLTVLHQDWLNGKEYKCKVSNKALPAPIEKTISKAKGQPREPQVYTLPPSREEMTKNQVSLTCLVKGFYPSDIAVEWESNGQPENNYKTTPPVLDSDGSFFLYSKLTVDKSRWQQGNVFSCSVMHEALHNHYTQKSLSLSPGK

SEQ ID NO: 29 - DNA, 1347 bp, Artificial Sequence
  source: /note="Description of Artificial Sequence: Synthetic polynucleotide"
caggtgcagctggtgcagtcaggcgccgaagtgaagaaacccggcgctagtgtgaaagtcagctgtaaagctagtgcctacaccttcacctctagctggatgcagtgggtcagacaggccccaggtcagggcctggagtggatgggcgagatcgaccctagcgataactacgctaactataatcagaagtttcagggtagagtcaccctgaccgtggacactagcactagcaccgcctatatggaactgtctagcctgagatcagaggacaccgccgtctactactgcgctagtggtagctacttctctaacttcttcgactactggggtcagggcaccctggtcaccgtgtctagcgctagcactaagggcccctccgtgttccctctggccccttccagcaagtctacctccggcggcacagctgctctgggctgcctggtcaaggactacttccctgagcctgtgacagtgtcctggaactctggcgccctgacctctggcgtgcacaccttccctgccgtgctgcagtcctccggcctgtactccctgtcctccgtggtcacagtgccttcaagcagcctgggcacccagacctatatctgcaacgtgaaccacaagccttccaacaccaaggtggacaagcgggtggagcctaagtcctgcgacaagacccacacctgtcctccctgccctgctcctgaagctgctggcggcccttctgtgttcctgttccctccaaagcccaaggacaccctgatgatctcccggacccctgaagtgacctgcgtggtggtggacgtgtcccacgaggatcctgaagtgaagttcaattggtacgtggacggcgtggaggtgcacaacgccaagaccaagcctcgggaggaacagtacaactccacctaccgggtggtgtccgtgctgaccgtgctgcaccaggactggctgaacggcaaagagtacaagtgcaaagtctccaacaaggccctgcctgcccctatcgaaaagacaatctccaaggccaagggccagcctagggaaccccaggtgtacaccctgccacccagccgggaggaaatgaccaagaaccaggtgtccctgacctgtctggtcaagggcttctacccttccgatatcgccgtggagtgggagtctaacggccagcctgagaacaactacaagaccacccctcctgtgctggactccgacggctccttcttcctgtactccaaactgaccgtggacaagtcccggtggcagcagggcaacgtgttctcctgctccgtgatgcacgaggccctgcacaaccactacacccagaagtccctgtccctgtctcccggcaag

SEQ ID NO: 30 - DNA, 321 bp, Artificial Sequence
  source: /note="Description of Artificial Sequence: Synthetic polynucleotide"
gagatcgtgatgactcagtcacccgctaccctgagcgtcagccctggcgagcgggctacactgagctgtaaagcctctcaggatatcggctctaacctgaactggctgcagcagaagcccggtcaggcccctagacggctgatctacgccgtgtctaatagaggccccggaatccccgctaggtttagcggctctaggtcaggttcagagtacaccctgactatctctagcctgcagtcagaggacttcgccgtctactactgcctgcagtacgcctctagcccctggaccttcggtcagggcactaaggtcgagattaag

SEQ ID NO: 31 - DNA, 642 bp, Artificial Sequence
  source: /note="Description of Artificial Sequence: Synthetic polynucleotide"
gagatcgtgatgactcagtcacccgctaccctgagcgtcagccctggcgagcgggctacactgagctgtaaagcctctcaggatatcggctctaacctgaactggctgcagcagaagcccggtcaggcccctagacggctgatctacgccgtgtctaatagaggccccggaatccccgctaggtttagcggctctaggtcaggttcagagtacaccctgactatctctagcctgcagtcagaggacttcgccgtctactactgcctgcagtacgcctctagcccctggaccttcggtcagggcactaaggtcgagattaagcgtacggtggccgctcccagcgtgttcatcttcccccccagcgacgagcagctgaagagcggcaccgccagcgtggtgtgcctgctgaacaacttctacccccgggaggccaaggtgcagtggaaggtggacaacgccctgcagagcggcaacagccaggagagcgtcaccgagcaggacagcaaggactccacctacagcctgagcagcaccctgaccctgagcaaggccgactacgagaagcataaggtgtacgcctgcgaggtgacccaccagggcctgtccagccccgtgaccaagagcttcaacaggggcgagtgc

SEQ ID NO: 32 - protein, 5 aa, Artificial Sequence
  source: /note="Description of Artificial Sequence: Synthetic peptide"
SSWMQ

SEQ ID NO: 33 - protein, 17 aa, Artificial Sequence
  source: /note="Description of Artificial Sequence: Synthetic peptide"
EIDPSDNYANYNQKFQG

SEQ ID NO: 34 - protein, 10 aa, Artificial Sequence
  source: /note="Description of Artificial Sequence: Synthetic peptide"
GSYFSNFFDY

SEQ ID NO: 35 - protein, 7 aa, Artificial Sequence
  source: /note="Description of Artificial Sequence: Synthetic peptide"
AYTFTSS

SEQ ID NO: 36 - protein, 6 aa, Artificial Sequence
  source: /note="Description of Artificial Sequence: Synthetic peptide"
DPSDNY

SEQ ID NO: 37 - protein, 10 aa, Artificial Sequence
  source: /note="Description of Artificial Sequence: Synthetic peptide"
GSYFSNFFDY

SEQ ID NO: 38 - protein, 119 aa, Artificial Sequence; identical to SEQ ID NO: 13
  source: /note="Description of Artificial Sequence: Synthetic polypeptide"

SEQ ID NO: 39 - DNA, 357 bp, Artificial Sequence; identical to SEQ ID NO: 14
  source: /note="Description of Artificial Sequence: Synthetic polynucleotide"

SEQ ID NO: 40 - protein, 449 aa, Artificial Sequence; identical to SEQ ID NO: 15
  source: /note="Description of Artificial Sequence: Synthetic polypeptide"

SEQ ID NO: 41 - DNA, 1347 bp, Artificial Sequence; identical to SEQ ID NO: 16
  source: /note="Description of Artificial Sequence: Synthetic polynucleotide"

SEQ ID NO: 42 - protein, 11 aa, Artificial Sequence
  source: /note="Description of Artificial Sequence: Synthetic peptide"
KASQDIGSNLN

SEQ ID NO: 43 - protein, 7 aa, Artificial Sequence
  source: /note="Description of Artificial Sequence: Synthetic peptide"
AASVREP

SEQ ID NO: 44 - protein, 9 aa, Artificial Sequence
  source: /note="Description of Artificial Sequence: Synthetic peptide"
LQYASSPWT

SEQ ID NO: 45 - protein, 7 aa, Artificial Sequence
  source: /note="Description of Artificial Sequence: Synthetic peptide"
SQDIGSN

SEQ ID NO: 46 - protein, 3 aa, Artificial Sequence
  source: /note="Description of Artificial Sequence: Synthetic peptide"
AAS

SEQ ID NO: 47 - protein, 6 aa, Artificial Sequence
  source: /note="Description of Artificial Sequence: Synthetic peptide"
YASSPW

SEQ ID NO: 48 - protein, 107 aa, Artificial Sequence
  source: /note="Description of Artificial Sequence: Synthetic polypeptide"
EIVMTQSPATLSVSPGERATLSCKASQDIGSNLNWLQQKPGQAPRRLIYAASVREPGIPARFSGSRSGSEYTLTISSLQSEDFAVYYCLQYASSPWTFGQGTKVEIK

SEQ ID NO: 49 - DNA, 321 bp, Artificial Sequence
  source: /note="Description of Artificial Sequence: Synthetic polynucleotide"
gagatcgtgatgacacagagccccgccaccctgtccgtgtctccaggcgaaagagccaccctgagctgcaaagccagccaggacatcggcagcaacctgaactggctgcagcagaaaccaggccaggcccccagaaggctgatctacgctgcttccgtccgtgagcctggcatccccgccagattttccggcagcagatccggcagcgagtacaccctgaccatcagcagcctgcagagcgaggacttcgccgtgtactactgcctgcagtacgccagcagcccctggacatttggccagggcaccaaggtggaaatcaag

SEQ ID NO: 50 - protein, 214 aa, Artificial Sequence
  source: /note="Description of Artificial Sequence: Synthetic polypeptide"
EIVMTQSPATLSVSPGERATLSCKASQDIGSNLNWLQQKPGQAPRRLIYAASVREPGIPARFSGSRSGSEYTLTISSLQSEDFAVYYCLQYASSPWTFGQGTKVEIKRTVAAPSVFIFPPSDEQLKSGTASVVCLLNNFYPREAKVQWKVDNALQSGNSQESVTEQDSKDSTYSLSSTLTLSKADYEKHKVYACEVTHQGLSSPVTKSFNRGEC

SEQ ID NO: 51 - DNA, 642 bp, Artificial Sequence
  source: /note="Description of Artificial Sequence: Synthetic polynucleotide"
gagatcgtgatgacacagagccccgccaccctgtccgtgtctccaggcgaaagagccaccctgagctgcaaagccagccaggacatcggcagcaacctgaactggctgcagcagaaaccaggccaggcccccagaaggctgatctacgctgcttccgtccgtgagcctggcatccccgccagattttccggcagcagatccggcagcgagtacaccctgaccatcagcagcctgcagagcgaggacttcgccgtgtactactgcctgcagtacgccagcagcccctggacatttggccagggcaccaaggtggaaatcaagcgtacggtggccgctcccagcgtgttcatcttcccccccagcgacgagcagctgaagagcggcaccgccagcgtggtgtgcctgctgaacaacttctacccccgggaggccaaggtgcagtggaaggtggacaacgccctgcagagcggcaacagccaggagagcgtcaccgagcaggacagcaaggactccacctacagcctgagcagcaccctgaccctgagcaaggccgactacgagaagcataaggtgtacgcctgcgaggtgacccaccagggcctgtccagccccgtgaccaagagcttcaacaggggcgagtgc

SEQ ID NO: 52 - protein, 5 aa, Artificial Sequence
  source: /note="Description of Artificial Sequence: Synthetic peptide"
SYTMH

SEQ ID NO: 53 - protein, 17 aa, Artificial Sequence
  source: /note="Description of Artificial Sequence: Synthetic peptide"
YINPSSGYTKYNQKFQG

SEQ ID NO: 54 - protein, 9 aa, Artificial Sequence
  source: /note="Description of Artificial Sequence: Synthetic peptide"
GWLLLAMDY

SEQ ID NO: 55 - protein, 7 aa, Artificial Sequence
  source: /note="Description of Artificial Sequence: Synthetic peptide"
GYTFTSY

SEQ ID NO: 56 - protein, 6 aa, Artificial Sequence
  source: /note="Description of Artificial Sequence: Synthetic peptide"
NPSSGY

SEQ ID NO: 57 - protein, 9 aa, Artificial Sequence
  source: /note="Description of Artificial Sequence: Synthetic peptide"
GWLLLAMDY

SEQ ID NO: 58 - protein, 118 aa, Artificial Sequence
  source: /note="Description of Artificial Sequence: Synthetic polypeptide"
QVQLVQSGAEVKKPGASVKVSCKASGYTFTSYTMHWVRQAPGQGLEWMGYINPSSGYTKYNQKFQGRVTMTADKSTSTAYMELSSLRSEDTAVYYCAEGWLLLAMDYWGQGTLVTVSS

SEQ ID NO: 59 - DNA, 354 bp, Artificial Sequence
  source: /note="Description of Artificial Sequence: Synthetic polynucleotide"
caggtgcagctggtgcagtctggcgccgaagtgaagaaaccaggcgccagcgtgaaggtgtcctgcaaggccagcggctacacctttaccagctacaccatgcactgggtgcgccaggctccaggccagggactggaatggatgggctacatcaaccccagcagcggctataccaagtacaaccagaaattccagggccgcgtgaccatgaccgccgacaagagcacaagcaccgcctacatggaactgagcagcctgcggagcgaggacaccgccgtgtactattgtgccgagggctggctgctgctggccatggattattggggccagggcaccctcgtgaccgtgtctagt

SEQ ID NO: 60 - protein, 448 aa, Artificial Sequence
  source: /note="Description of Artificial Sequence: Synthetic polypeptide"
QVQLVQSGAEVKKPGASVKVSCKASGYTFTSYTMHWVRQAPGQGLEWMGYINPSSGYTKYNQKFQGRVTMTADKSTSTAYMELSSLRSEDTAVYYCAEGWLLLAMDYWGQGTLVTVSSASTKGPSVFPLAPSSKSTSGGTAALGCLVKDYFPEPVTVSWNSGALTSGVHTFPAVLQSSGLYSLSSVVTVPSSSLGTQTYICNVNHKPSNTKVDKRVEPKSCDKTHTCPPCPAPELLGGPSVFLFPPKPKDTLMISRTPEVTCVVVDVSHEDPEVKFNWYVDGVEVHNAKTKPREEQYNSTYRVVSVLTVLHQDWLNGKEYKCKVSNKALPAPIEKTISKAKGQPREPQVYTLPPSREEMTKNQVSLTCLVKGFYPSDIAVEWESNGQPENNYKTTPPVLDSDGSFFLYSKLTVDKSRWQQGNVFSCSVMHEALHNHYTQKSLSLSPGK

SEQ ID NO: 61 - DNA, 1344 bp, Artificial Sequence
  source: /note="Description of Artificial Sequence: Synthetic polynucleotide"
caggtgcagctggtgcagtctggcgccgaagtgaagaaaccaggcgccagcgtgaaggtgtcctgcaaggccagcggctacacctttaccagctacaccatgcactgggtgcgccaggctccaggccagggactggaatggatgggctacatcaaccccagcagcggctataccaagtacaaccagaaattccagggccgcgtgaccatgaccgccgacaagagcacaagcaccgcctacatggaactgagcagcctgcggagcgaggacaccgccgtgtactattgtgccgagggctggctgctgctggccatggattattggggccagggcaccctcgtgaccgtgtctagtgctagcaccaagggccccagcgtgttccccctggcccccagcagcaagagcaccagcggcggcacagccgccctgggctgcctggtgaaggactacttccccgagcccgtgaccgtgtcctggaacagcggagccctgacctccggcgtgcacaccttccccgccgtgctgcagagcagcggcctgtacagcctgtccagcgtggtgacagtgcccagcagcagcctgggcacccagacctacatctgcaacgtgaaccacaagcccagcaacaccaaggtggacaagagagtggagcccaagagctgcgacaagacccacacctgccccccctgcccagccccagagctgctgggcggaccctccgtgttcctgttcccccccaagcccaaggacaccctgatgatcagcaggacccccgaggtgacctgcgtggtggtggacgtgagccacgaggacccagaggtgaagttcaactggtacgtggacggcgtggaggtgcacaacgccaagaccaagcccagagaggagcagtacaacagcacctacagggtggtgtccgtgctgaccgtgctgcaccaggactggctgaacggcaaggaatacaagtgcaaggtctccaacaaggccctgccagcccccatcgaaaagaccatcagcaaggccaagggccagccacgggagccccaggtgtacaccctgcccccctcccgggaggagatgaccaagaaccaggtgtccctgacctgtctggtgaagggcttctaccccagcgacatcgccgtggagtgggagagcaacggccagcccgagaacaactacaagaccacccccccagtgctggacagcgacggcagcttcttcctgtacagcaagctgaccgtggacaagtccaggtggcagcagggcaacgtgttcagctgcagcgtgatgcacgaggccctgcacaaccactacacccagaagagcctgagcctgtcccccggcaag

SEQ ID NO: 62 - protein, 14 aa, Artificial Sequence
  source: /note="Description of Artificial Sequence: Synthetic peptide"
RSSTGAVTTSNYAI

SEQ ID NO: 63 - protein, 7 aa, Artificial Sequence
  source: /note="Description of Artificial Sequence: Synthetic peptide"
GTNNRAP

SEQ ID NO: 64 - protein, 9 aa, Artificial Sequence
  source: /note="Description of Artificial Sequence: Synthetic peptide"
ALWYSDHWV

SEQ ID NO: 65 - protein, 10 aa, Artificial Sequence
  source: /note="Description of Artificial Sequence: Synthetic peptide"
STGAVTTSNY

SEQ ID NO: 66 - protein, 3 aa, Artificial Sequence
  source: /note="Description of Artificial Sequence: Synthetic peptide"
GTN

SEQ ID NO: 67 - protein, 6 aa, Artificial Sequence
  source: /note="Description of Artificial Sequence: Synthetic peptide"
WYSDHW

SEQ ID NO: 68 - protein, 110 aa, Artificial Sequence
  source: /note="Description of Artificial Sequence: Synthetic polypeptide"
EAVVTQSPATLSLSPGERATLSCRSSTGAVTTSNYAIWVQEKPGQAPRGLIGGTNNRAPGIPARFSGSLSGDDATLTISSLQPEDFAVYFCALWYSDHWVFGQGTKVEIK

SEQ ID NO: 69 - DNA, 330 bp, Artificial Sequence
  source: /note="Description of Artificial Sequence: Synthetic polynucleotide"
gaagccgtcgtgacacagagccctgccaccctgtcactgagccctggcgaaagagccaccctgagctgcagatctagcaccggcgctgtgaccaccagcaactacgccatctgggtgcaggaaaagcccggccaggctcccagaggactgatcggcggcaccaacaatagagcccctggcatccccgccagattcagcggatctctgtctggcgacgacgccacactgaccatcagcagcctgcagcccgaggacttcgccgtgtacttctgcgccctgtggtacagcgaccactgggtgttcggccagggcaccaaggtggaaatcaag

SEQ ID NO: 70 - protein, 217 aa, Artificial Sequence
  source: /note="Description of Artificial Sequence: Synthetic polypeptide"
EAVVTQSPATLSLSPGERATLSCRSSTGAVTTSNYAIWVQEKPGQAPRGLIGGTNNRAPGIPARFSGSLSGDDATLTISSLQPEDFAVYFCALWYSDHWVFGQGTKVEIKRTVAAPSVFIFPPSDEQLKSGTASVVCLLNNFYPREAKVQWKVDNALQSGNSQESVTEQDSKDSTYSLSSTLTLSKADYEKHKVYACEVTHQGLSSPVTKSFNRGEC

SEQ ID NO: 71 - DNA, 651 bp, Artificial Sequence
  source: /note="Description of Artificial Sequence: Synthetic polynucleotide"
gaagccgtcgtgacacagagccctgccaccctgtcactgagccctggcgaaagagccaccctgagctgcagatctagcaccggcgctgtgaccaccagcaactacgccatctgggtgcaggaaaagcccggccaggctcccagaggactgatcggcggcaccaacaatagagcccctggcatccccgccagattcagcggatctctgtctggcgacgacgccacactgaccatcagcagcctgcagcccgaggacttcgccgtgtacttctgcgccctgtggtacagcgaccactgggtgttcggccagggcaccaaggtggaaatcaagcgtacggtggccgctcccagcgtgttcatcttcccccccagcgacgagcagctgaagagcggcaccgccagcgtggtgtgcctgctgaacaacttctacccccgggaggccaaggtgcagtggaaggtggacaacgccctgcagagcggcaacagccaggagagcgtcaccgagcaggacagcaaggactccacctacagcctgagcagcaccctgaccctgagcaaggccgactacgagaagcataaggtgtacgcctgcgaggtgacccaccagggcctgtccagccccgtgaccaagagcttcaacaggggcgagtgc

SEQ ID NO: 72 - protein, 5 aa, Artificial Sequence
  source: /note="Description of Artificial Sequence: Synthetic peptide"
NYWIT

SEQ ID NO: 73 - protein, 17 aa, Artificial Sequence
  source: /note="Description of Artificial Sequence: Synthetic peptide"
DFYPGGGSTNYNAKLQG

SEQ ID NO: 74 - protein, 10 aa, Artificial Sequence
  source: /note="Description of Artificial Sequence: Synthetic peptide"
SPPQVAPFDY

SEQ ID NO: 75 - protein, 7 aa, Artificial Sequence
  source: /note="Description of Artificial Sequence: Synthetic peptide"
GYTFNNY

SEQ ID NO: 76 - protein, 6 aa, Artificial Sequence
  source: /note="Description of Artificial Sequence: Synthetic peptide"
YPGGGS

SEQ ID NO: 77 - protein, 10 aa, Artificial Sequence
  source: /note="Description of Artificial Sequence: Synthetic peptide"
SPPQVAPFDY

SEQ ID NO: 78 - protein, 119 aa, Artificial Sequence
  source: /note="Description of Artificial Sequence: Synthetic polypeptide"
QVQLVQSGAEVKKPGASVKVSCKASGYTFNNYWITWVRQAPGQGLEWMGDFYPGGGSTNYNAKLQGRVTLTVDTSTSTAYMELRSLRSDDTAVYYCARSPPQVAPFDYWGQGTLVTVSS

SEQ ID NO: 79 - DNA, 357 bp, Artificial Sequence
  source: /note="Description of Artificial Sequence: Synthetic polynucleotide"
caggtgcagctggtgcagtctggcgccgaagtgaagaaaccaggcgccagcgtgaaggtgtcctgcaaggccagcggctacacctttaacaactactggatcacctgggtgcgccaggcccctggacagggactggaatggatgggcgacttctaccctggcggcggcagcaccaactacaacgccaagctgcagggcagagtgaccctgaccgtggacaccagcacctccaccgcctacatggaactgcggagcctgagaagcgacgacaccgccgtgtattactgcgctagaagccctcctcaggtggcccccttcgattattggggccagggcacactcgtgaccgtgtcctct

SEQ ID NO: 80 - protein, 449 aa, Artificial Sequence
  source: /note="Description of Artificial Sequence: Synthetic polypeptide"
QVQLVQSGAEVKKPGASVKVSCKASGYTFNNYWITWVRQAPGQGLEWMGDFYPGGGSTNYNAKLQGRVTLTVDTSTSTAYMELRSLRSDDTAVYYCARSPPQVAPFDYWGQGTLVTVSSASTKGPSVFPLAPSSKSTSGGTAALGCLVKDYFPEPVTVSWNSGALTSGVHTFPAVLQSSGLYSLSSVVTVPSSSLGTQTYICNVNHKPSNTKVDKRVEPKSCDKTHTCPPCPAPELLGGPSVFLFPPKPKDTLMISRTPEVTCVVVDVSHEDPEVKFNWYVDGVEVHNAKTKPREEQYNSTYRVVSVLTVLHQDWLNGKEYKCKVSNKALPAPIEKTISKAKGQPREPQVYTLPPSREEMTKNQVSLTCLVKGFYPSDIAVEWESNGQPENNYKTTPPVLDSDGSFFLYSKLTVDKSRWQQGNVFSCSVMHEALHNHYTQKSLSLSPGK

SEQ ID NO: 81 - DNA, 1347 bp, Artificial Sequence
  source: /note="Description of Artificial Sequence: Synthetic polynucleotide"
caggtgcagctggtgcagtctggcgccgaagtgaagaaaccaggcgccagcgtgaaggtgtcctgcaaggccagcggctacacctttaacaactactggatcacctgggtgcgccaggcccctggacagggactggaatggatgggcgacttctaccctggcggcggcagcaccaactacaacgccaagctgcagggcagagtgaccctgaccgtggacaccagcacctccaccgcctacatggaactgcggagcctgagaagcgacgacaccgccgtgtattactgcgctagaagccctcctcaggtggcccccttcgattattggggccagggcacactcgtgaccgtgtcctctgctagcaccaagggccccagcgtgttccccctggcccccagcagcaagagcaccagcggcggcacagccgccctgggctgcctggtgaaggactacttccccgagcccgtgaccgtgtcctggaacagcggagccctgacctccggcgtgcacaccttccccgccgtgctgcagagcagcggcctgtacagcctgtccagcgtggtgacagtgcccagcagcagcctgggcacccagacctacatctgcaacgtgaaccacaagcccagcaacaccaaggtggacaagagagtggagcccaagagctgcgacaagacccacacctgccccccctgcccagccccagagctgctgggcggaccctccgtgttcctgttcccccccaagcccaaggacaccctgatgatcagcaggacccccgaggtgacctgcgtggtggtggacgtgagccacgaggacccagaggtgaagttcaactggtacgtggacggcgtggaggtgcacaacgccaagaccaagcccagagaggagcagtacaacagcacctacagggtggtgtccgtgctgaccgtgctgcaccaggactggctgaacggcaaggaatacaagtgcaaggtctccaacaaggccctgccagcccccatcgaaaagaccatcagcaaggccaagggccagccacgggagccccaggtgtacaccctgcccccctcccgggaggagatgaccaagaaccaggtgtccctgacctgtctggtgaagggcttctaccccagcgacatcgccgtggagtgggagagcaacggccagcccgagaacaactacaagaccacccccccagtgctggacagcgacggcagcttcttcctgtacagcaagctgaccgtggacaagtccaggtggcagcagggcaacgtgttcagctgcagcgtgatgcacgaggccctgcacaaccactacacccagaagagcctgagcctgtcccccggcaag

SEQ ID NO: 82 - protein, 11 aa, Artificial Sequence
  source: /note="Description of Artificial Sequence: Synthetic peptide"
QASDYIYHWLG

SEQ ID NO: 83 - protein, 7 aa, Artificial Sequence
  source: /note="Description of Artificial Sequence: Synthetic peptide"
GASGLET

SEQ ID NO: 84 - protein, 9 aa, Artificial Sequence
  source: /note="Description of Artificial Sequence: Synthetic peptide"
QQYWSTPWT

SEQ ID NO: 85 - protein, 7 aa, Artificial Sequence
  source: /note="Description of Artificial Sequence: Synthetic peptide"
SDYIYHW

SEQ ID NO: 86 - protein, 3 aa, Artificial Sequence
  source: /note="Description of Artificial Sequence: Synthetic peptide"
GAS

SEQ ID NO: 87 - protein, 6 aa, Artificial Sequence
  source: /note="Description of Artificial Sequence: Synthetic peptide"
YWSTPW

SEQ ID NO: 88 - protein, 107 aa, Artificial Sequence
  source: /note="Description of Artificial Sequence: Synthetic polypeptide"
DIQMTQSPSSLSASVGDRVTITCQASDYIYHWLGWYQQKPGKAPKLLISGASGLETGVPSRFSGSGSGKDYTFTISSLQPEDIATYYCQQYWSTPWTFGQGTKLEIK

SEQ ID NO: 89 - DNA, 321 bp, Artificial Sequence
  source: /note="Description of Artificial Sequence: Synthetic polynucleotide"
gacatccagatgacccagagccccagcagcctgtctgccagcgtgggcgacagggtgaccatcacctgtcaggccagcgactacatctaccactggctgggctggtatcagcagaagcccggcaaggcccccaagctgctgattagcggagcctccggtctggaaaccggcgtgccaagcagattttccggcagcggctccggcaaggactacaccttcaccatcagctccctgcagcccgaggatatcgccacctactactgccagcagtactggtccaccccctggacctttggccagggcaccaagctggaaatcaag

SEQ ID NO: 90 - protein, 214 aa, Artificial Sequence
  source: /note="Description of Artificial Sequence: Synthetic polypeptide"
DIQMTQSPSSLSASVGDRVTITCQASDYIYHWLGWYQQKPGKAPKLLISGASGLETGVPSRFSGSGSGKDYTFTISSLQPEDIATYYCQQYWSTPWTFGQGTKLEIKRTVAAPSVFIFPPSDEQLKSGTASVVCLLNNFYPREAKVQWKVDNALQSGNSQESVTEQDSKDSTYSLSSTLTLSKADYEKHKVYACEVTHQGLSSPVTKSFNRGEC

SEQ ID NO: 91 - DNA, 642 bp, Artificial Sequence
  source: /note="Description of Artificial Sequence: Synthetic polynucleotide"
gacatccagatgacccagagccccagcagcctgtctgccagcgtgggcgacagggtgaccatcacctgtcaggccagcgactacatctaccactggctgggctggtatcagcagaagcccggcaaggcccccaagctgctgattagcggagcctccggtctggaaaccggcgtgccaagcagattttccggcagcggctccggcaaggactacaccttcaccatcagctccctgcagcccgaggatatcgccacctactactgccagcagtactggtccaccccctggacctttggccagggcaccaagctggaaatcaagcgtacggtggccgctcccagcgtgttcatcttcccccccagcgacgagcagctgaagagcggcaccgccagcgtggtgtgcctgctgaacaacttctacccccgggaggccaaggtgcagtggaaggtggacaacgccctgcagagcggcaacagccaggagagcgtcaccgagcaggacagcaaggactccacctacagcctgagcagcaccctgaccctgagcaaggccgactacgagaagcataaggtgtacgcctgcgaggtgacccaccagggcctgtccagccccgtgaccaagagcttcaacaggggcgagtgc

SEQ ID NO: 92 - protein, 5 aa, Artificial Sequence
  source: /note="Description of Artificial Sequence: Synthetic peptide"
NYWIT

SEQ ID NO: 93 - protein, 17 aa, Artificial Sequence
  source: /note="Description of Artificial Sequence: Synthetic peptide"
DFYPGGGNTNYNAKLQG

SEQ ID NO: 94 - protein, 10 aa, Artificial Sequence
  source: /note="Description of Artificial Sequence: Synthetic peptide"
SPPQVAPFDY

SEQ ID NO: 95 - protein, 7 aa, Artificial Sequence
  source: /note="Description of Artificial Sequence: Synthetic peptide"
GYTFTNY

SEQ ID NO: 96 - protein, 6 aa, Artificial Sequence
  source: /note="Description of Artificial Sequence: Synthetic peptide"
YPGGGN

SEQ ID NO: 97 - protein, 10 aa, Artificial Sequence
  source: /note="Description of Artificial Sequence: Synthetic peptide"
SPPQVAPFDY

SEQ ID NO: 98 - protein, 119 aa, Artificial Sequence
  source: /note="Description of Artificial Sequence: Synthetic polypeptide"
QVQLVQSGAEVKKPGASVKVSCKASGYTFTNYWITWVRQAPGQGLEWMGDFYPGGGNTNYNAKLQGRVTLTVDTSTSTAYMELRSLRSDDTAVYYCARSPPQVAPFDYWGQGTLVTVSS

SEQ ID NO: 99 - DNA, 357 bp, Artificial Sequence
  source: /note="Description of Artificial Sequence: Synthetic polynucleotide"
caggtgcagctggtgcagtctggcgccgaagtgaagaaaccaggcgccagcgtgaaggtgtcctgcaaggccagcggctacacctttaccaactactggatcacctgggtgcgccaggcccctggacagggactggaatggatgggcgacttctaccctggcggcggcaacaccaactacaacgccaagctgcagggcagagtgaccctgaccgtggacaccagcacctccaccgcctacatggaactgcggagcctgagaagcgacgacaccgccgtgtattactgcgctagaagccctcctcaggtggcccccttcgattattggggccagggcacactcgtgaccgtgtcctct

SEQ ID NO: 100 - protein, 449 aa, Artificial Sequence
  source: /note="Description of Artificial Sequence: Synthetic polypeptide"
QVQLVQSGAEVKKPGASVKVSCKASGYTFTNYWITWVRQAPGQGLEWMGDFYPGGGNTNYNAKLQGRVTLTVDTSTSTAYMELRSLRSDDTAVYYCARSPPQVAPFDYWGQGTLVTVSSASTKGPSVFPLAPSSKSTSGGTAALGCLVKDYFPEPVTVSWNSGALTSGVHTFPAVLQSSGLYSLSSVVTVPSSSLGTQTYICNVNHKPSNTKVDKRVEPKSCDKTHTCPPCPAPELLGGPSVFLFPPKPKDTLMISRTPEVTCVVVDVSHEDPEVKFNWYVDGVEVHNAKTKPREEQYNSTYRVVSVLTVLHQDWLNGKEYKCKVSNKALPAPIEKTISKAKGQPREPQVYTLPPSREEMTKNQVSLTCLVKGFYPSDIAVEWESNGQPENNYKTTPPVLDSDGSFFLYSKLTVDKSRWQQGNVFSCSVMHEALHNHYTQKSLSLSPGK

SEQ ID NO: 101 - DNA, 1347 bp, Artificial Sequence
  source: /note="Description of Artificial Sequence: Synthetic polynucleotide"
caggtgcagctggtgcagtctggcgccgaagtgaagaaaccaggcgccagcgtgaaggtgtcctgcaaggccagcggctacacctttaccaactactggatcacctgggtgcgccaggcccctggacagggactggaatggatgggcgacttctaccctggcggcggcaacaccaactacaacgccaagctgcagggcagagtgaccctgaccgtggacaccagcacctccaccgcctacatggaactgcggagcctgagaagcgacgacaccgccgtgtattactgcgctagaagccctcctcaggtggcccccttcgattattggggccagggcacactcgtgaccgtgtcctctgctagcaccaagggccccagcgtgttccccctggcccccagcagcaagagcaccagcggcggcacagccgccctgggctgcctggtgaaggactacttccccgagcccgtgaccgtgtcctggaacagcggagccctgacctccggcgtgcacaccttccccgccgtgctgcagagcagcggcctgtacagcctgtccagcgtggtgacagtgcccagcagcagcctgggcacccagacctacatctgcaacgtgaaccacaagcccagcaacaccaaggtggacaagagagtggagcccaagagctgcgacaagacccacacctgccccccctgcccagccccagagctgctgggcggaccctccgtgttcctgttcccccccaagcccaaggacaccctgatgatcagcaggacccccgaggtgacctgcgtggtggtggacgtgagccacgaggacccagaggtgaagttcaactggtacgtggacggcgtggaggtgcacaacgccaagaccaagcccagagaggagcagtacaacagcacctacagggtggtgtccgtgctgaccgtgctgcaccaggactggctgaacggcaaggaatacaagtgcaaggtctccaacaaggccctgccagcccccatcgaaaagaccatcagcaaggccaagggccagccacgggagccccaggtgtacaccctgcccccctcccgggaggagatgaccaagaaccaggtgtccctgacctgtctggtgaagggcttctaccccagcgacatcgccgtggagtgggagagcaacggccagcccgagaacaactacaagaccacccccccagtgctggacagcgacggcagcttcttcctgtacagcaagctgaccgtggacaagtccaggtggcagcagggcaacgtgttcagctgcagcgtgatgcacgaggccctgcacaaccactacacccagaagagcctgagcctgtcccccggcaag

SEQ ID NO: 102 - protein, 11 aa, Artificial Sequence
  source: /note="Description of Artificial Sequence: Synthetic peptide"
QASEYIYNWLG

SEQ ID NO: 103 - protein, 7 aa, Artificial Sequence
  source: /note="Description of Artificial Sequence: Synthetic peptide"
GASGLET

SEQ ID NO: 104 - protein, 9 aa, Artificial Sequence
  source: /note="Description of Artificial Sequence: Synthetic peptide"
QQYWSTPWT

SEQ ID NO: 105 - protein, 7 aa, Artificial Sequence
  source: /note="Description of Artificial Sequence: Synthetic peptide"
SEYIYNW

SEQ ID NO: 106 - protein, 3 aa, Artificial Sequence
  source: /note="Description of Artificial Sequence: Synthetic peptide"
GAS

SEQ ID NO: 107 - protein, 6 aa, Artificial Sequence
  source: /note="Description of Artificial Sequence: Synthetic peptide"
YWSTPW

SEQ ID NO: 108 - protein, 107 aa, Artificial Sequence
  source: /note="Description of Artificial Sequence: Synthetic polypeptide"
DIQMTQSPSSLSASVGDRVTITCQASEYIYNWLGWYQQKPGKAPKLLISGASGLETGVPSRFSGSGSGKDYTFTISSLQPEDIATYYCQQYWSTPWTFGQGTKLEIK

SEQ ID NO: 109 - DNA, 321 bp, Artificial Sequence
  source: /note="Description of Artificial Sequence: Synthetic polynucleotide"
gacatccagatgacccagagccccagcagcctgtctgccagcgtgggcgacagggtgaccatcacctgtcaggccagcgaatacatctacaactggctgggctggtatcagcagaagcccggcaaggcccccaagctgctgattagcggagcctccggtctggaaaccggcgtgccaagcagattttccggcagcggctccggcaaggactacaccttcaccatcagctccctgcagcccgaggatatcgccacctactactgccagcagtactggtccaccccctggacctttggccagggcaccaagctggaaatcaag

SEQ ID NO: 110 - protein, 214 aa, Artificial Sequence
  source: /note="Description of Artificial Sequence: Synthetic polypeptide"
DIQMTQSPSSLSASVGDRVTITCQASEYIYNWLGWYQQKPGKAPKLLISGASGLETGVPSRFSGSGSGKDYTFTISSLQPEDIATYYCQQYWSTPWTFGQGTKLEIKRTVAAPSVFIFPPSDEQLKSGTASVVCLLNNFYPREAKVQWKVDNALQSGNSQESVTEQDSKDSTYSLSSTLTLSKADYEKHKVYACEVTHQGLSSPVTKSFNRGEC

SEQ ID NO: 111 - DNA, 642 bp, Artificial Sequence
  source: /note="Description of Artificial Sequence: Synthetic polynucleotide"
gacatccagatgacccagagccccagcagcctgtctgccagcgtgggcgacagggtgaccatcacctgtcaggccagcgaatacatctacaactggctgggctggtatcagcagaagcccggcaaggcccccaagctgctgattagcggagcctccggtctggaaaccggcgtgccaagcagattttccggcagcggctccggcaaggactacaccttcaccatcagctccctgcagcccgaggatatcgccacctactactgccagcagtactggtccaccccctggacctttggccagggcaccaagctggaaatcaagcgtacggtggccgctcccagcgtgttcatcttcccccccagcgacgagcagctgaagagcggcaccgccagcgtggtgtgcctgctgaacaacttctacccccgggaggccaaggtgcagtggaaggtggacaacgccctgcagagcggcaacagccaggagagcgtcaccgagcaggacagcaaggactccacctacagcctgagcagcaccctgaccctgagcaaggccgactacgagaagcataaggtgtacgcctgcgaggtgacccaccagggcctgtccagccccgtgaccaagagcttcaacaggggcgagtgc

SEQ ID NO: 112 - protein, 5 aa, Artificial Sequence
  source: /note="Description of Artificial Sequence: Synthetic peptide"
SFWIT

SEQ ID NO: 113 - protein, 17 aa, Artificial Sequence
  source: /note="Description of Artificial Sequence: Synthetic peptide"
DIYPGGATTNYNEKLQG

SEQ ID NO: 114 - protein, 10 aa, Artificial Sequence
  source: /note="Description of Artificial Sequence: Synthetic peptide"
SPPQVGPFDY

SEQ ID NO: 115 - protein, 7 aa, Artificial Sequence
  source: /note="Description of Artificial Sequence: Synthetic peptide"
GYTFTSF

SEQ ID NO: 116 - protein, 6 aa, Artificial Sequence
  source: /note="Description of Artificial Sequence: Synthetic peptide"
YPGGAT

SEQ ID NO: 117 - protein, 10 aa, Artificial Sequence
  source: /note="Description of Artificial Sequence: Synthetic peptide"
SPPQVGPFDY

SEQ ID NO: 118 - protein, 119 aa, Artificial Sequence
  source: /note="Description of Artificial Sequence: Synthetic polypeptide"
QVQLVQSGAEVKKPGASVKVSCKASGYTFTSFWITWVRQAPGQGLEWMGDIYPGGATTNYNEKLQGRVTLTVDTSTSTAYMELRSLRSDDTAVYYCARSPPQVGPFDYWGQGTLVTVSS

SEQ ID NO: 119 - DNA, 357 bp, Artificial Sequence
  source: /note="Description of Artificial Sequence: Synthetic polynucleotide"
caggtgcagctggtgcagtctggcgccgaagtgaagaaaccaggcgccagcgtgaaggtgtcctgcaaggccagcggctataccttcaccagcttttggatcacctgggtgcgccaggcccctggacagggactggaatggatgggcgacatctaccctggcggcgccaccaccaactacaacgagaagctgcagggcagagtgaccctgaccgtggacaccagcacctccaccgcctacatggaactgcggagcctgagaagcgacgacaccgccgtgtactactgcgctagaagccctcctcaggtgggccccttcgattattggggccagggcacactcgtgaccgtgtcctct

SEQ ID NO: 120 - protein, 449 aa, Artificial Sequence
  source: /note="Description of Artificial Sequence: Synthetic polypeptide"
QVQLVQSGAEVKKPGASVKVSCKASGYTFTSFWITWVRQAPGQGLEWMGDIYPGGATTNYNEKLQGRVTLTVDTSTSTAYMELRSLRSDDTAVYYCARSPPQVGPFDYWGQGTLVTVSSASTKGPSVFPLAPSSKSTSGGTAALGCLVKDYFPEPVTVSWNSGALTSGVHTFPAVLQSSGLYSLSSVVTVPSSSLGTQTYICNVNHKPSNTKVDKRVEPKSCDKTHTCPPCPAPELLGGPSVFLFPPKPKDTLMISRTPEVTCVVVDVSHEDPEVKFNWYVDGVEVHNAKTKPREEQYNSTYRVVSVLTVLHQDWLNGKEYKCKVSNKALPAPIEKTISKAKGQPREPQVYTLPPSREEMTKNQVSLTCLVKGFYPSDIAVEWESNGQPENNYKTTPPVLDSDGSFFLYSKLTVDKSRWQQGNVFSCSVMHEALHNHYTQKSLSLSPGK

SEQ ID NO: 121 - DNA, 1347 bp, Artificial Sequence
  source: /note="Description of Artificial Sequence: Synthetic polynucleotide"
caggtgcagctggtgcagtctggcgccgaagtgaagaaaccaggcgccagcgtgaaggtgtcctgcaaggccagcggctataccttcaccagcttttggatcacctgggtgcgccaggcccctggacagggactggaatggatgggcgacatctaccctggcggcgccaccaccaactacaacgagaagctgcagggcagagtgaccctgaccgtggacaccagcacctccaccgcctacatggaactgcggagcctgagaagcgacgacaccgccgtgtactactgcgctagaagccctcctcaggtgggccccttcgattattggggccagggcacactcgtgaccgtgtcctctgctagcaccaagggccccagcgtgttccccctggcccccagcagcaagagcaccagcggcggcacagccgccctgggctgcctggtgaaggactacttccccgagcccgtgaccgtgtcctggaacagcggagccctgacctccggcgtgcacaccttccccgccgtgctgcagagcagcggcctgtacagcctgtccagcgtggtgacagtgcccagcagcagcctgggcacccagacctacatctgcaacgtgaaccacaagcccagcaacaccaaggtggacaagagagtggagcccaagagctgcgacaagacccacacctgccccccctgcccagccccagagctgctgggcggaccctccgtgttcctgttcccccccaagcccaaggacaccctgatgatcagcaggacccccgaggtgacctgcgtggtggtggacgtgagccacgaggacccagaggtgaagttcaactggtacgtggacggcgtggaggtgcacaacgccaagaccaagcccagagaggagcagtacaacagcacctacagggtggtgtccgtgctgaccgtgctgcaccaggactggctgaacggcaaggaatacaagtgcaaggtctccaacaaggccctgccagcccccatcgaaaagaccatcagcaaggccaagggccagccacgggagccccaggtgtacaccctgcccccctcccgggaggagatgaccaagaaccaggtgtccctgacctgtctggtgaagggcttctaccccagcgacatcgccgtggagtgggagagcaacggccagcccgagaacaactacaagaccacccccccagtgctggacagcgacggcagcttcttcctgtacagcaagctgaccgtggacaagtccaggtggcagcagggcaacgtgttcagctgcagcgtgatgcacgaggccctgcacaaccactacacccagaagagcctgagcctgtcccccggcaag

SEQ ID NO: 122 - protein, 11 aa, Artificial Sequence
  source: /note="Description of Artificial Sequence: Synthetic peptide"
QASDYIYHWLA

SEQ ID NO: 123 - protein, 7 aa, Artificial Sequence
  source: /note="Description of Artificial Sequence: Synthetic peptide"
GASSLET

SEQ ID NO: 124 - protein, 9 aa, Artificial Sequence
  source: /note="Description of Artificial Sequence: Synthetic peptide"
QQYWSIPWT

SEQ ID NO: 125 - protein, 7 aa, Artificial Sequence
  source: /note="Description of Artificial Sequence: Synthetic peptide"
SDYIYHW

SEQ ID NO: 126 - protein, 3 aa, Artificial Sequence
  source: /note="Description of Artificial Sequence: Synthetic peptide"
GAS

SEQ ID NO: 127 - protein, 6 aa, Artificial Sequence
  source: /note="Description of Artificial Sequence: Synthetic peptide"
YWSIPW

SEQ ID NO: 128 - protein, 107 aa, Artificial Sequence
  source: /note="Description of Artificial Sequence: Synthetic polypeptide"
DIQMTQSPSSLSASVGDRVTITCQASDYIYHWLAWYQQKPGKAPKLLISGASSLETGVPSRFSGSGSGKDYTFTISSLQPEDIATYYCQQYWSIPWTFGQGTKLEIK

SEQ ID NO: 129 - DNA, 321 bp, Artificial Sequence
  source: /note="Description of Artificial Sequence: Synthetic polynucleotide"
gacatccagatgacccagagccccagcagcctgtctgccagcgtgggcgacagagtgaccatcacctgtcaggccagcgactacatctaccactggctggcctggtatcagcagaagcccggcaaggcccccaagctgctgattagcggagcctccagtctggaaaccggcgtgccaagcagattttccggcagcggctccggcaaggactacaccttcaccatcagctccctgcagcccgaggatatcgccacctactactgccagcagtactggtccatcccctggacctttggccagggcaccaagctggaaatcaag

SEQ ID NO: 130 - protein, 214 aa, Artificial Sequence
  source: /note="Description of Artificial Sequence: Synthetic polypeptide"
DIQMTQSPSSLSASVGDRVTITCQASDYIYHWLAWYQQKPGKAPKLLISGASSLETGVPSRFSGSGSGKDYTFTISSLQPEDIATYYCQQYWSIPWTFGQGTKLEIKRTVAAPSVFIFPPSDEQLKSGTASVVCLLNNFYPREAKVQWKVDNALQSGNSQESVTEQDSKDSTYSLSSTLTLSKADYEKHKVYACEVTHQGLSSPVTKSFNRGEC

SEQ ID NO: 131 - DNA, 642 bp, Artificial Sequence
  source: /note="Description of Artificial Sequence: Synthetic polynucleotide"
gacatccagatgacccagagccccagcagcctgtctgccagcgtgggcgacagagtgaccatcacctgtcaggccagcgactacatctaccactggctggcctggtatcagcagaagcccggcaaggcccccaagctgctgattagcggagcctccagtctggaaaccggcgtgccaagcagattttccggcagcggctccggcaaggactacaccttcaccatcagctccctgcagcccgaggatatcgccacctactactgccagcagtactggtccatcccctggacctttggccagggcaccaagctggaaatcaagcgtacggtggccgctcccagcgtgttcatcttcccccccagcgacgagcagctgaagagcggcaccgccagcgtggtgtgcctgctgaacaacttctacccccgggaggccaaggtgcagtggaaggtggacaacgccctgcagagcggcaacagccaggagagcgtcaccgagcaggacagcaaggactccacctacagcctgagcagcaccctgaccctgagcaaggccgactacgagaagcataaggtgtacgcctgcgaggtgacccaccagggcctgtccagccccgtgaccaagagcttcaacaggggcgagtgc

SEQ ID NO: 132 - protein, 5 aa, Artificial Sequence
  source: /note="Description of Artificial Sequence: Synthetic peptide"
SFWIT

SEQ ID NO: 133 - protein, 17 aa, Artificial Sequence
  source: /note="Description of Artificial Sequence: Synthetic peptide"
DIYPGGANTNYNEKLQG

SEQ ID NO: 134 - protein, 10 aa, Artificial Sequence
  source: /note="Description of Artificial Sequence: Synthetic peptide"
SPPQVGPFDY

SEQ ID NO: 135 - protein, 7 aa, Artificial Sequence
  source: /note="Description of Artificial Sequence: Synthetic peptide"
GYTFTSF

SEQ ID NO: 136 - protein, 6 aa, Artificial Sequence
  source: /note="Description of Artificial Sequence: Synthetic peptide"
YPGGAN

SEQ ID NO: 137 - protein, 10 aa, Artificial Sequence
  source: /note="Description of Artificial Sequence: Synthetic peptide"
SPPQVGPFDY

SEQ ID NO: 138 - protein, 119 aa, Artificial Sequence
  source: /note="Description of Artificial Sequence: Synthetic polypeptide"
QVQLVQSGAEVKKPGASVKVSCKASGYTFTSFWITWVRQAPGQGLEWMGDIYPGGANTNYNEKLQGRVTLTVDTSTSTAYMELRSLRSDDTAVYYCARSPPQVGPFDYWGQGTLVTVSS

SEQ ID NO: 139 - DNA, 357 bp, Artificial Sequence
  source: /note="Description of Artificial Sequence: Synthetic polynucleotide"
caggtgcagctggtgcagtctggcgccgaagtgaagaaaccaggcgccagcgtgaaggtgtcctgcaaggccagcggctataccttcaccagcttttggatcacctgggtgcgccaggcccctggacagggactggaatggatgggcgacatctaccctggcggcgccaacaccaactacaacgagaagctgcagggcagagtgaccctgaccgtggacaccagcacctccaccgcctacatggaactgcggagcctgagaagcgacgacaccgccgtgtactactgcgctagaagccctcctcaggtgggccccttcgattattggggccagggcacactcgtgaccgtgtcctct

SEQ ID NO: 140 - protein, 449 aa, Artificial Sequence
  source: /note="Description of Artificial Sequence: Synthetic polypeptide"
QVQLVQSGAEVKKPGASVKVSCKASGYTFTSFWITWVRQAPGQGLEWMGDIYPGGANTNYNEKLQGRVTLTVDTSTSTAYMELRSLRSDDTAVYYCARSPPQVGPFDYWGQGTLVTVSSASTKGPSVFPLAPSSKSTSGGTAALGCLVKDYFPEPVTVSWNSGALTSGVHTFPAVLQSSGLYSLSSVVTVPSSSLGTQTYICNVNHKPSNTKVDKRVEPKSCDKTHTCPPCPAPELLGGPSVFLFPPKPKDTLMISRTPEVTCVVVDVSHEDPEVKFNWYVDGVEVHNAKTKPREEQYNSTYRVVSVLTVLHQDWLNGKEYKCKVSNKALPAPIEKTISKAKGQPREPQVYTLPPSREEMTKNQVSLTCLVKGFYPSDIAVEWESNGQPENNYKTTPPVLDSDGSFFLYSKLTVDKSRWQQGNVFSCSVMHEALHNHYTQKSLSLSPGK

SEQ ID NO: 141 - DNA, 1347 bp, Artificial Sequence
  source: /note="Description of Artificial Sequence: Synthetic polynucleotide"
caggtgcagctggtgcagtctggcgccgaagtgaagaaaccaggcgccagcgtgaaggtgtcctgcaaggccagcggctataccttcaccagcttttggatcacctgggtgcgccaggcccctggacagggactggaatggatgggcgacatctaccctggcggcgccaacaccaactacaacgagaagctgcagggcagagtgaccctgaccgtggacaccagcacctccaccgcctacatggaactgcggagcctgagaagcgacgacaccgccgtgtactactgcgctagaagccctcctcaggtgggccccttcgattattggggccagggcacactcgtgaccgtgtcctctgctagcaccaagggccccagcgtgttccccctggcccccagcagcaagagcaccagcggcggcacagccgccctgggctgcctggtgaaggactacttccccgagcccgtgaccgtgtcctggaacagcggagccctgacctccggcgtgcacaccttccccgccgtgctgcagagcagcggcctgtacagcctgtccagcgtggtgacagtgcccagcagcagcctgggcacccagacctacatctgcaacgtgaaccacaagcccagcaacaccaaggtggacaagagagtggagcccaagagctgcgacaagacccacacctgccccccctgcccagccccagagctgctgggcggaccctccgtgttcctgttcccccccaagcccaaggacaccctgatgatcagcaggacccccgaggtgacctgcgtggtggtggacgtgagccacgaggacccagaggtgaagttcaactggtacgtggacggcgtggaggtgcacaacgccaagaccaagcccagagaggagcagtacaacagcacctacagggtggtgtccgtgctgaccgtgctgcaccaggactggctgaacggcaaggaatacaagtgcaaggtctccaacaaggccctgccagcccccatcgaaaagaccatcagcaaggccaagggccagccacgggagccccaggtgtacaccctgcccccctcccgggaggagatgaccaagaaccaggtgtccctgacctgtctggtgaagggcttctaccccagcgacatcgccgtggagtgggagagcaacggccagcccgagaacaactacaagaccacccccccagtgctggacagcgacggcagcttcttcctgtacagcaagctgaccgtggacaagtccaggtggcagcagggcaacgtgttcagctgcagcgtgatgcacgaggccctgcacaaccactacacccagaagagcctgagcctgtcccccggcaag

SEQ ID NO: 142 - protein, 11 aa, Artificial Sequence
  source: /note="Description of Artificial Sequence: Synthetic peptide"
QASEYIINWLA

SEQ ID NO: 143 - protein, 7 aa, Artificial Sequence
  source: /note="Description of Artificial Sequence: Synthetic peptide"
GATGLET

SEQ ID NO: 144 - protein, 9 aa, Artificial Sequence
  source: /note="Description of Artificial Sequence: Synthetic peptide"
QQYWSIPWT

SEQ ID NO: 145 - protein, 7 aa, Artificial Sequence
  source: /note="Description of Artificial Sequence: Synthetic peptide"
SEYIINW

SEQ ID NO: 146 - protein, 3 aa, Artificial Sequence
  source: /note="Description of Artificial Sequence: Synthetic peptide"
GAT

SEQ ID NO: 147 - protein, 6 aa, Artificial Sequence
  source: /note="Description of Artificial Sequence: Synthetic peptide"
YWSIPW

SEQ ID NO: 148 - protein, 107 aa, Artificial Sequence
  source: /note="Description of Artificial Sequence: Synthetic polypeptide"
DIQMTQSPSSLSASVGDRVTITCQASEYIINWLAWYQQKPGKAPKLLISGATGLETGVPSRFSGSGSGKDYTFTISSLQPEDIATYYCQQYWSIPWTFGQGTKLEIK

SEQ ID NO: 149 - DNA, 321 bp, Artificial Sequence
  source: /note="Description of Artificial Sequence: Synthetic polynucleotide"
gacatccagatgacccagagccccagcagcctgtctgccagcgtgggcgacagagtgaccatcacctgtcaggccagcgaatacatcataaactggctggcctggtatcagcagaagcccggcaaggcccccaagctgctgattagcggagccaccggtctggaaaccggcgtgccaagcagattttccggcagcggctccggcaaggactacaccttcaccatcagctccctgcagcccgaggatatcgccacctactactgccagcagtactggtccatcccctggacctttggccagggcaccaagctggaaatcaag

SEQ ID NO: 150 - protein, 214 aa, Artificial Sequence
  source: /note="Description of Artificial Sequence: Synthetic polypeptide"
DIQMTQSPSSLSASVGDRVTITCQASEYIINWLAWYQQKPGKAPKLLISGATGLETGVPSRFSGSGSGKDYTFTISSLQPEDIATYYCQQYWSIPWTFGQGTKLEIKRTVAAPSVFIFPPSDEQLKSGTASVVCLLNNFYPREAKVQWKVDNALQSGNSQESVTEQDSKDSTYSLSSTLTLSKADYEKHKVYACEVTHQGLSSPVTKSFNRGEC

SEQ ID NO: 151 - DNA, 642 bp, Artificial Sequence
  source: /note="Description of Artificial Sequence: Synthetic polynucleotide"
gacatccagatgacccagagccccagcagcctgtctgccagcgtgggcgacagagtgaccatcacctgtcaggccagcgaatacatcataaactggctggcctggtatcagcagaagcccggcaaggcccccaagctgctgattagcggagccaccggtctggaaaccggcgtgccaagcagattttccggcagcggctccggcaaggactacaccttcaccatcagctccctgcagcccgaggatatcgccacctactactgccagcagtactggtccatcccctggacctttggccagggcaccaagctggaaatcaagcgtacggtggccgctcccagcgtgttcatcttcccccccagcgacgagcagctgaagagcggcaccgccagcgtggtgtgcctgctgaacaacttctacccccgggaggccaaggtgcagtggaaggtggacaacgccctgcagagcggcaacagccaggagagcgtcaccgagcaggacagcaaggactccacctacagcctgagcagcaccctgaccctgagcaaggccgactacgagaagcataaggtgtacgcctgcgaggtgacccaccagggcctgtccagccccgtgaccaagagcttcaacaggggcgagtgc

SEQ ID NO: 152 - protein, 24 aa, Homo sapiens
MKTFILLLWVLLLWVIFLLPGATA

SEQ ID NO: 153 - protein, 9 aa, Artificial Sequence
  source: /note="Description of Artificial Sequence: Synthetic peptide"
DYKDDDDKH

SEQ ID NO: 154 - protein, 6 aa, Artificial Sequence
  source: /note="Description of Artificial Sequence: Synthetic 6xHis tag"
HHHHHH

SEQ ID NO: 155 - protein, 17 aa, Artificial Sequence
  source: /note="Description of Artificial Sequence: Synthetic peptide"
GGGLNDIFEAQKIEWHE

SEQ ID NO: 156 - protein, 438 aa, Artificial Sequence
  source: /note="Description of Artificial Sequence: Synthetic polypeptide"
MKTFILLLWVLLLWVIFLLPGATAQPGPVQSKSPRFASWDEMNVLAHGLLQLGQGLREHAERTRSQLSALERRLSACGSACQGTEGSTDLPLAPESRVDPEVLHSLQTQLKAQNSRIQQLFHKVAQQQRHLEKQHLRIQHLQSQFGLLDHKHLDHEVAKPARRKRLPEMAQPVDPAHNVSRLHRLPRDCQELFQVGERQSGLFEIQPQGSPPFLVNCKMTSDGGWTVIQRRHDGSVDFNRPWEAYKAGFGDPHGEFWLGLEKVHSITGDRNSRLAVQLRDWDGNAELLQFSVHLGGEDTAYSLQLTAPVAGQLGATTVPPSGLSVPFSTWDQDHDLRRDKNCAKSLSGGWWFGTCSHSNLNGQYFRSIPQQRQKLKKGIFWKTWRGRYYPLQATTMLIQPMAAEAASDYKDDDDKHHHHHHGGGLNDIFEAQKIEWHE

SEQ ID NO: 157 - protein, 232 aa, Artificial Sequence
  source: /note="Description of Artificial Sequence: Synthetic polypeptide"
MKTFILLLWVLLLWVIFLLPGATAQPGPVQSKSPRFASWDEMNVLAHGLLQLGQGLREHAERTRSQLSALERRLSACGSACQGTEGSTDLPLAPESRVDPEVLHSLQTQLKAQNSRIQQLFHKVAQQQRHLEKQHLRIQHLQSQFGLLDHKHLDHEVAKPARRKRLPEMAQPVDPAHNVSRLHRLPRDYKDDDDKHHHHHHDYKDDDDKHHHHHHGGGLNDIFEAQKIEWHE

SEQ ID NO: 158 - DNA, 19 bp, Artificial Sequence
  source: /note="Description of Artificial Sequence: Synthetic primer"
atccccgctcccaggctac

SEQ ID NO: 159 - DNA, 24 bp, Artificial Sequence
  source: /note="Description of Artificial Sequence: Synthetic primer"
cagcaaggagtgaagctccatgcc

SEQ ID NO: 160 - protein, 438 aa, Artificial Sequence
  source: /note="Description of Artificial Sequence: Synthetic polypeptide"
MKTFILLLWVLLLWVIFLLPGATAQPGPVQSKSPRFASWDEMNVLAHGLLQLGQGLREHAERTRSQLNALERRLSACGSACQGTEGSTALPLAPESRVDPEVLHSLQTQLKAQNSRIQQLFHKVAQQQRHLEKQHLRIQRLQSQVGLLDPKHLDHEVAKPARRKRRPEMAQPVDSAHNASRLHRLPRDCQELFEDGERQSGLFEIQPQGSPPFLVNCKMTSDGGWTVIQRRHDGSVDFNRPWEAYKAGFGDPQGEFWLGLEKVHSITGDRNSRLAVQLQDWDGNAESLQFSVHLGGEDTAYSLQLTEPVASQLGATTVPPSGLSVPFSTWDQDHDLRRDKNCAKSLSGGWWFGTCSHSNLNGQYFRSIPQQRQELKKGIFWKTWRGRYYPLQATTMLIQPTAAEAASDYKDDDDKHHHHHHGGGLNDIFEAQKIEWHE

SEQ ID NO: 161 - protein, 218 aa, Artificial Sequence
  source: /note="Description of Artificial Sequence: Synthetic polypeptide"
MKTFILLLWVLLLWVIFLLPGATAQPGPVQSKSPRFASWDEMNVLAHGLLQLGQGLREHAERTRSQLNALERRLSACGSACQGTEGSTALPLAPESRVDPEVLHSLQTQLKAQNSRIQQLFHKVAQQQRHLEKQHLRIQRLQSQVGLLDPKHLDHEVAKPARRKRRPEMAQPVDSAHNASRLHRLPRDYKDDDDKHHHHHHGGGLNDIFEAQKIEWHE

SEQ ID NO: 162 - protein, 442 aa, Artificial Sequence
  source: /note="Description of Artificial Sequence: Synthetic polypeptide"
MKTFILLLWVLLLWVIFLLPGATAQPRPAQPEPPRFASWDEMNLLAHGLLQLGHGLREHVERTRGQLGALERRMAACGNACQGPKGKDAPFKDSEDRVPEGQTPETLQSLQTQLKAQNSKIQQLFQKVAQQQRYLSKQNLRIQNLQSQIDLLAPTHLDNGVDKTSRGKRLPKMTQLIGLTPNATHLHRPPRDCQELFQEGERHSGLFQIQPLGSPPFLVNCEMTSDGGWTVIQRRLNGSVDFNQSWEAYKDGFGDPQGEFWLGLEKMHSITGNRGSQLAVQLQDWDGNAKLLQFPIHLGGEDTAYSLQLTEPTANELGATNVSPNGLSLPFSTWDQDHDLRGDLNCAKSLSGGWWFGTCSHSNLNGQYFHSIPRQRQERKKGIFWKTWKGRYYPLQATTLLIQPMEATAASDYKDDDDKHHHHHHGGGLNDIFEAQKIEWHE

SEQ ID NO: 163 - protein, 440 aa, Artificial Sequence
  source: /note="Description of Artificial Sequence: Synthetic polypeptide"
MKTFILLLWVLLLWVIFLLPGATAQPQGRPAQPEPPRFASWDEMNLLAHGLLQLGHGLREHVERTRGQLGALERRMAACGNACQGPKGTDPKDRVPEGQAPETLQSLQTQLKAQNSKIQQLFQKVAQQQRYLSKQNLRIQNLQSQIDLLTPTHLDNGVDKTSRGKRLPKMAQLIGLTPNATRLHRPPRDCQELFQEGERHSGLFQIQPLGSPPFLVNCEMTSDGGWTVIQRRLNGSVDFNQSWEAYKDGFGDPQGEFWLGLEKMHSITGDRGSQLAVQLQDWDGNAKLLQFPIHLGGEDTAYSLQLTEPTANELGATNVSPNGLSLPFSTWDQDHDLRGDLNCAKSLSGGWWFGTCSHSNLNGQYFHSIPRQRQQRKKGIFWKTWKGRYYPLQATTLLIQPMEATAASDYKDDDDKHHHHHHGGGLNDIFEAQKIEWHET

SEQ ID NO: 164 - protein, 501 aa, Artificial Sequence
  source: /note="Description of Artificial Sequence: Synthetic polypeptide"
MKTFILLLWVLLLWVIFLLPGATAQPSRIDQDNSSFDSLSPEPKSRFAMLDDVKILANGLLQLGHGLKDFVHKTKGQINDIFQKLNIFDQSFYDLSLQTSEIKEEEKELRRTTYKLQVKNEEVKNMSLELNSKLESLLEEKILLQQKVKYLEEQLTNLIQNQPETPEHPEVTSLKTFVEKQDNSIKDLLQTVEDQYKQLNQQHSQIKEIENQLRRTSIQEPTEISLSSKPRAPRTTPFLQLNEIRNVKHDGIPAECTTIYNRGEHTSGMYAIRPSNSQVFHVYCDVISGSPWTLIQHRIDGSQNFNETWENYKYGFGRLDGEFWLGLEKIYSIVKQSNYVLRIELEDWKDNKHYIEYSFYLGNHETNYTLHLVAITGNVPNAIPENKDLVFSTWDHKAKGHFNCPEGYSGGWWWHDECGENNLNGKYNKPRAKSKPERRRGLSWKSQNGRLYSIKSTKMLIHPTDSESFEDYKDDDDKHHHHHHGGGLNDIFEAQKIEWHE

SEQ ID NO: 165 - protein, 10 aa, Homo sapiens
GPVQSKSPRF

SEQ ID NO: 166 - protein, 11 aa, Homo sapiens
VQSKSPRFASW

SEQ ID NO: 167 - protein, 8 aa, Homo sapiens
NVLAHGLL

SEQ ID NO: 168 - protein, 10 aa, Homo sapiens
NVLAHGLLQL

SEQ ID NO: 169 - protein, 8 aa, Homo sapiens
LAHGLLQL

SEQ ID NO: 170 - protein, 13 aa, Homo sapiens
NVLAHGLLQLGQG

SEQ ID NO: 171 - protein, 14 aa, Homo sapiens
NVLAHGLLQLGQGL

SEQ ID NO: 172 - protein, 16 aa, Homo sapiens
NVLAHGLLQLGQGLRE

SEQ ID NO: 173 - protein, 25 aa, Homo sapiens
NVLAHGLLQLGQGLREHAERTRSQL

SEQ ID NO: 174 - protein, 27 aa, Homo sapiens
NVLAHGLLQLGQGLREHAERTRSQLSA

SEQ ID NO: 175 - protein, 23 aa, Homo sapiens
LAHGLLQLGQGLREHAERTRSQL

SEQ ID NO: 176 - protein, 13 aa, Homo sapiens
AHGLLQLGQGLRE

SEQ ID NO: 177 - protein, 22 aa, Homo sapiens
AHGLLQLGQGLREHAERTRSQL

SEQ ID NO: 178 - protein, 18 aa, Homo sapiens
LQLGQGLREHAERTRSQL

SEQ ID NO: 179 - protein, 15 aa, Homo sapiens
GQGLREHAERTRSQL

SEQ ID NO: 180 - protein, 32 aa, Homo sapiens
LERRLSACGSACQTEGSTDLPAPESRVDPEVL

SEQ ID NO: 181 - protein, 25 aa, Homo sapiens
CGSACQTEGSTDLPAPESRVDPEVL

SEQ ID NO: 182 - protein, 16 aa, Homo sapiens
STDLPAPESRVDPEVL

SEQ ID NO: 183 - protein, 7 aa, Homo sapiens
RVDPEVL

SEQ ID NO: 184 - protein, 7 aa, Homo sapiens
HSLQTQL

SEQ ID NO: 185 - protein, 10 aa, Homo sapiens
KAQNSRIQQL

SEQ ID NO: 186 - protein, 26 aa, Homo sapiens
KAQNSRIQQLFHKVAQQQRHLEKQHL

SEQ ID NO: 187 - protein, 16 aa, Homo sapiens
FHKVAQQQRHLEKQHL

SEQ ID NO: 188 - protein, 7 aa, Homo sapiens
QSQFGLL

SEQ ID NO: 189 - protein, 12 aa, Homo sapiens
FGLLDHKHLDHE

SEQ ID NO: 190 - protein, 26 aa, Homo sapiens
LERRLSACGSACQTEGSTDLPLAPES

SEQ ID NO: 191 - protein, 15 aa, Artificial Sequence
  source: /note="Description of Artificial Sequence: Synthetic peptide"
GPVQSKSPRFASWDE

SEQ ID NO: 192 - protein, 15 aa, Artificial Sequence
  source: /note="Description of Artificial Sequence: Synthetic peptide"
QSKSPRFASWDEMNV

SEQ ID NO: 193 - protein, 15 aa, Artificial Sequence
  source: /note="Description of Artificial Sequence: Synthetic peptide"
SPRFASWDEMNVLAH

SEQ ID NO: 194 - protein, 15 aa, Artificial Sequence
  source: /note="Description of Artificial Sequence: Synthetic peptide"
FASWDEMNVLAHGLL

SEQ ID NO: 195 - protein, 15 aa, Artificial Sequence
  source: /note="Description of Artificial Sequence: Synthetic peptide"
WDEMNVLAHGLLQLG

SEQ ID NO: 196 - protein, 15 aa, Artificial Sequence
  source: /note="Description of Artificial Sequence: Synthetic peptide"
MNVLAHGLLQLGQGL

SEQ ID NO: 197 - protein, 15 aa, Artificial Sequence
  source: /note="Description of Artificial Sequence: Synthetic peptide"
LAHGLLQLGQGLREH

SEQ ID NO: 198 - protein, 15 aa, Artificial Sequence
  source: /note="Description of Artificial Sequence: Synthetic peptide"
GLLQLGQGLREHAER

SEQ ID NO: 199 - protein, 15 aa, Artificial Sequence
  source: /note="Description of Artificial Sequence: Synthetic peptide"
QLGQGLREHAERTRS

SEQ ID NO: 200 - protein, 15 aa, Artificial Sequence
  source: /note="Description of Artificial Sequence: Synthetic peptide"
QGLREHAERTRSQLS

SEQ ID NO: 201 - protein, 15 aa, Artificial Sequence
  source: /note="Description of Artificial Sequence: Synthetic peptide"
REHAERTRSQLSALE

SEQ ID NO: 202 - protein, 15 aa, Artificial Sequence
  source: /note="Description of Artificial Sequence: Synthetic peptide"
AERTRSQLSALERRL

SEQ ID NO: 203 - protein, 15 aa, Artificial Sequence
  source: /note="Description of Artificial Sequence: Synthetic peptide"
TRSQLSALERRLSAS

SEQ ID NO: 204 - protein, 15 aa, Artificial Sequence
  source: /note="Description of Artificial Sequence: Synthetic peptide"
QLSALERRLSASGSA

SEQ ID NO: 205 - protein, 15 aa, Artificial Sequence
  source: /note="Description of Artificial Sequence: Synthetic peptide"
ALERRLSASGSASQG

SEQ ID NO: 206 - protein, 15 aa, Artificial Sequence
  source: /note="Description of Artificial Sequence: Synthetic peptide"
RRLSASGSASQGTEG

SEQ ID NO: 207 - protein, 15 aa, Artificial Sequence
  source: /note="Description of Artificial Sequence: Synthetic peptide"
SASGSASQGTEGSTD

SEQ ID NO: 208 - protein, 15 aa, Artificial Sequence
  source: /note="Description of Artificial Sequence: Synthetic peptide"
GSASQGTEGSTDLPL

SEQ ID NO: 209 - protein, 15 aa, Artificial Sequence
  source: /note="Description of Artificial Sequence: Synthetic peptide"
SQGTEGSTDLPLAPE

SEQ ID NO: 210 - protein, 15 aa, Artificial Sequence
  source: /note="Description of Artificial Sequence: Synthetic peptide"
TEGSTDLPLAPESRV

SEQ ID NO: 211 - protein, 15 aa, Artificial Sequence
  source: /note="Description of Artificial Sequence: Synthetic peptide"
STDLPLAPESRVDPE

SEQ ID NO: 212 - protein, 15 aa, Artificial Sequence
  source: /note="Description of Artificial Sequence: Synthetic peptide"
LPLAPESRVDPEVLH

SEQ ID NO: 213 - protein, 15 aa, Artificial Sequence
  source: /note="Description of Artificial Sequence: Synthetic peptide"
APESRVDPEVLHSLQ

SEQ ID NO: 214 - protein, 15 aa, Artificial Sequence
  source: /note="Description of Artificial Sequence: Synthetic peptide"
SRVDPEVLHSLQTQL

SEQ ID NO: 215 - protein, 15 aa, Artificial Sequence
  source: /note="Description of Artificial Sequence: Synthetic peptide"
DPEVLHSLQTQLKAQ

SEQ ID NO: 216 - protein, 15 aa, Artificial Sequence
  source: /note="Description of Artificial Sequence: Synthetic peptide"
VLHSLQTQLKAQNSR

SEQ ID NO: 217 - protein, 15 aa, Artificial Sequence
  source: /note="Description of Artificial Sequence: Synthetic peptide"
SLQTQLKAQNSRIQQ

SEQ ID NO: 218 - protein, 15 aa, Artificial Sequence
  source: /note="Description of Artificial Sequence: Synthetic peptide"
TQLKAQNSRIQQLFH

SEQ ID NO: 219 - protein, 15 aa, Artificial Sequence
  source: /note="Description of Artificial Sequence: Synthetic peptide"
KAQNSRIQQLFHKVA

SEQ ID NO: 220 - protein, 15 aa, Artificial Sequence
  source: /note="Description of Artificial Sequence: Synthetic peptide"
NSRIQQLFHKVAQQQ

SEQ ID NO: 221 - protein, 15 aa, Artificial Sequence
  source: /note="Description of Artificial Sequence: Synthetic peptide"
IQQLFHKVAQQQRHL

SEQ ID NO: 222 - protein, 15 aa, Artificial Sequence
  source: /note="Description of Artificial Sequence: Synthetic peptide"
LFHKVAQQQRHLEKQ

SEQ ID NO: 223 - protein, 15 aa, Artificial Sequence
  source: /note="Description of Artificial Sequence: Synthetic peptide"
KVAQQQRHLEKQHLR

SEQ ID NO: 224 - protein, 15 aa, Artificial Sequence
  source: /note="Description of Artificial Sequence: Synthetic peptide"
QQQRHLEKQHLRIQH

SEQ ID NO: 225 - protein, 15 aa, Artificial Sequence
  source: /note="Description of Artificial Sequence: Synthetic peptide"
RHLEKQHLRIQHLQS

SEQ ID NO: 226 - protein, 15 aa, Artificial Sequence
  source: /note="Description of Artificial Sequence: Synthetic peptide"
EKQHLRIQHLQSQFG

SEQ ID NO: 227 - protein, 15 aa, Artificial Sequence
  source: /note="Description of Artificial Sequence: Synthetic peptide"
HLRIQHLQSQFGLLD

SEQ ID NO: 228 - protein, 15 aa, Artificial Sequence
  source: /note="Description of Artificial Sequence: Synthetic peptide"
IQHLQSQFGLLDHKH

SEQ ID NO: 229 - protein, 15 aa, Artificial Sequence
  source: /note="Description of Artificial Sequence: Synthetic peptide"
LQSQFGLLDHKHLDH

SEQ ID NO: 230 - protein, 15 aa, Artificial Sequence
  source: /note="Description of Artificial Sequence: Synthetic peptide"
QFGLLDHKHLDHEVA

SEQ ID NO: 231 - protein, 15 aa, Artificial Sequence
  source: /note="Description of Artificial Sequence: Synthetic peptide"
LLDHKHLDHEVAKPA

SEQ ID NO: 232 - protein, 15 aa, Artificial Sequence
  source: /note="Description of Artificial Sequence: Synthetic peptide"
HKHLDHEVAKPARRK

SEQ ID NO: 233 - protein, 15 aa, Artificial Sequence
  source: /note="Description of Artificial Sequence: Synthetic peptide"
KHLDHEVAKPARRKR